European Patent Specification EP 3 390 625 B1, published September 6, 2023. Title: POLYPEPTIDES WITH ENDOGLUCANASE ACTIVITY AND USES THEREOF. Applicant: Danisco US Inc. The sequence listing filed with the application follows.

SEQUENCE LISTING (29 sequences)

SEQ ID NO: 1 - protein, 316 aa, Staphylotrichum coccosporum
MRSSPVLRTALAAALPLAALAADGKSTRYWDCCKPSCSWPGKASVNQPVFACSANFQRISDPNVKSGCDGGSAYACADQTPWAVNDNFSYGFAATSISGGNEASWCCGCYELTFTSGPVAGKTMVVQSTSTGGDLGTNHFDLAMPGGGVGIFDGCSPQFGGLAGDRYGGVSSRSQCDSFPAALKPGCYWRFDWFKNADNPTFTFRQVQCPSELVARTGCRRNDDGNFPVFTPPSGGQSSSSSSSSSAKPTSTSTSTTSTKATSTTSTASSQTSSSTGGGCAAQRWAQCGGIGFSGCTTCVSGTTCNKQNDWYSQCL

SEQ ID NO: 2 - protein, 238 aa, Madurella mycetomatis
MHSAPVLRAALIATLPLAAHAASGSGQSTRYWDCCKPSCSWPGKAPVNQPVFACDANFQRINDFGATSGCDGGSAYSCADHAPWAINDNLSYGFAATALSGETESSWCCACYALTFTSGPVAGKTMVVQSTSTGGDLGSNHFDLNIPGGGVGLFDGCTPQFGGLPGAQYGGISDRSQCSSFPSQLQPGCNWRFDWFMNADNPSFTFDQVQCPDELVARTGCRRSDDANFPAFSPPSRL

SEQ ID NO: 3 - DNA, 951 bp, Staphylotrichum coccosporum
atgcgttcctcccccgtcctccgcacggccctggccgctgccctccccctggccgccctcgctgccgatggcaagtcgacccgctactgggactgttgcaagccgtcgtgctcgtggcccggcaaggcctcggtgaaccagcccgtcttcgcctgcagcgccaacttccagcgcatcagcgaccccaacgtcaagtcgggctgcgacggcggctccgcctacgcctgcgccgaccagaccccgtgggccgtcaacgacaacttctcgtacggcttcgccgccacgtccatctcgggcggcaacgaggcctcgtggtgctgtggctgctacgagctgaccttcacctcgggccccgtcgctggcaagaccatggttgtccagtccacctcgaccggcggcgacctcggcaccaaccacttcgacctggccatgcccggtggtggtgtcggcatcttcgacggctgctcgccccagttcggcggcctcgccggcgaccgctacggcggcgtctcgtcgcgcagccagtgcgactcgttccccgccgccctcaagcccggctgctactggcgcttcgactggttcaagaacgccgacaacccgaccttcaccttccgccaggtccagtgcccgtcggagctcgtcgcccgcaccggctgccgccgcaacgacgacggcaacttccccgtcttcacccctccctcgggcggtcagtcctcctcgtcttcctcctccagcagcgccaagcccacctccacctccacctcgaccacctccaccaaggctacctccaccacctcgaccgcctccagccagacctcgtcgtccaccggcggcggctgcgccgcccagcgctgggcgcagtgcggcggcatcgggttctcgggctgcaccacgtgcgtcagcggcaccacctgcaacaagcagaacgactggtactcgcagtgcctttga

SEQ ID NO: 4 - protein, 316 aa, Staphylotrichum coccosporum; identical to SEQ ID NO: 1

SEQ ID NO: 5 - protein, 295 aa, Staphylotrichum coccosporum
ADGKSTRYWDCCKPSCSWPGKASVNQPVFACSANFQRISDPNVKSGCDGGSAYACADQTPWAVNDNFSYGFAATSISGGNEASWCCGCYELTFTSGPVAGKTMVVQSTSTGGDLGTNHFDLAMPGGGVGIFDGCSPQFGGLAGDRYGGVSSRSQCDSFPAALKPGCYWRFDWFKNADNPTFTFRQVQCPSELVARTGCRRNDDGNFPVFTPPSGGQSSSSSSSSSAKPTSTSTSTTSTKATSTTSTASSQTSSSTGGGCAAQRWAQCGGIGFSGCTTCVSGTTCNKQNDWYSQCL

SEQ ID NO: 6 - protein, 214 aa, Staphylotrichum coccosporum
ADGKSTRYWDCCKPSCSWPGKASVNQPVFACSANFQRISDPNVKSGCDGGSAYACADQTPWAVNDNFSYGFAATSISGGNEASWCCGCYELTFTSGPVAGKTMVVQSTSTGGDLGTNHFDLAMPGGGVGIFDGCSPQFGGLAGDRYGGVSSRSQCDSFPAALKPGCYWRFDWFKNADNPTFTFRQVQCPSELVARTGCRRNDDGNFPVFTPPSG

SEQ ID NO: 7 - protein, 338 aa, artificial sequence
  variant of BPN' protein
AQSVPYGVSQIKAPALHSQGYTGSNVKVAVIDSGIDSSHPDLKVAGGASMVPSETNPFQDNNSHGTHVAGTVAALNNSIGVLGVAPSASLYAVKVLGADGSGQYSWIINGIEWAIANNMDVINMSLGGPSGSAALKAAVDKAVASGVVVVAAAGNEGTSGSSSTVGYPGKYPSVIAVGAVDSSNQRASFSSVGPELDVMAPGVSIQSTLPGNKYGALNGTSMASPHVAGAAALILSKHPNWTNTQVRSSLENTTTKLGDSFYYGKGLINVQAAAQKSFPEVVGKTVDQAREYFTLHYPQYDVYFLPEGSPVTLDLRYNRVKVFYNPGTNVVNHVPHVG

SEQ ID NO: 8 - protein, 295 aa, artificial sequence
  mature form of the STCE1-A142P variant
ADGKSTRYWDCCKPSCSWPGKASVNQPVFACSANFQRISDPNVKSGCDGGSAYACADQTPWAVNDNFSYGFAATSISGGNEASWCCGCYELTFTSGPVAGKTMVVQSTSTGGDLGTNHFDLAMPGGGVGIFDGCSPQFGGLPGDRYGGVSSRSQCDSFPAALKPGCYWRFDWFKNADNPTFTFRQVQCPSELVARTGCRRNDDGNFPVFTPPSGGQSSSSSSSSSAKPTSTSTSTTSTKATSTTSTASSQTSSSTGGGCAAQRWAQCGGIGFSGCTTCVSGTTCNKQNDWYSQCL

SEQ ID NO: 9 - DNA, 1060 bp, Humicola insolens
ggatccaagatgcgttcctcccccctcctcccgtccgccgttgtggccgccctgccggtgttggcccttgccgctgatggcaggtccacccgctactgggactgctgcaagccttcgtgcggctgggccaagaaggctcccgtgaaccagcctgtcttttcctgcaacgccaacttccagcgtatcacggacttcgacgccaagtccggctgcgagccgggcggtgtcgcctactcgtgcgccgaccagaccccatgggctgtgaacgacgacttcgcgctcggttttgctgccacctctattgccggcagcaatgaggcgggctggtgctgcgcctgctacgagctcaccttcacatccggtcctgttgctggcaagaagatggtcgtccagtccaccagcactggcggtgatcttggcagcaaccacttcgatctcaacatccccggcggcggcgtcggcatcttcgacggatgcactccccagttcggcggtctgcccggccagcgctacggcggcatctcgtcccgcaacgagtgcgatcggttccccgacgccctcaagcccggctgctactggcgcttcgactggttcaagaacgccgacaatccgagcttcagcttccgtcaggtccagtgcccagccgagctcgtcgctcgcaccggatgccgccgcaacgacgacggcaacttccctgccgtccagatcccctccagcagcaccagctctccggtcaaccagcctaccagcaccagcaccacgtccacctccaccacctcgagcccgccagtccagcctacgactcccagcggctgcactgctgagaggtgggctcagtgcggcggcaatggctggagcggctgcaccacctgcgtcgctggcagcacttgcacgaagattaatgactggtaccatcagtgcctgtagacgcagggcagcttgagggccttactggtggccgcaacgaaatgacactcccaatcactgtattagttcttgtacataatttcgtcatccctccagggattgtcacataaatgcaatgaggaacaatgagtac

SEQ ID NO: 10 - protein, 305 aa, Humicola insolens
MRSSPLLPSAVVAALPVLALAADGRSTRYWDCCKPSCGWAKKAPVNQPVFSCNANFQRITDFDAKSGCEPGGVAYSCADQTPWAVNDDFALGFAATSIAGSNEAGWCCACYELTFTSGPVAGKKMVVQSTSTGGDLGSNHFDLNIPGGGVGIFDGCTPQFGGLPGQRYGGISSRNECDRFPDALKPGCYWRFDWFKNADNPSFSFRQVQCPAELVARTGCRRNDDGNFPAVQIPSSSTSSPVNQPTSTSTTSTSTTSSPPVQPTTPSGCTAERWAQCGGNGWSGCTTCVAGSTCTKINDWYHQCL

SEQ ID NO: 11 - protein, 284 aa, Humicola insolens
ADGRSTRYWDCCKPSCGWAKKAPVNQPVFSCNANFQRITDFDAKSGCEPGGVAYSCADQTPWAVNDDFALGFAATSIAGSNEAGWCCACYELTFTSGPVAGKKMVVQSTSTGGDLGSNHFDLNIPGGGVGIFDGCTPQFGGLPGQRYGGISSRNECDRFPDALKPGCYWRFDWFKNADNPSFSFRQVQCPAELVARTGCRRNDDGNFPAVQIPSSSTSSPVNQPTSTSTTSTSTTSSPPVQPTTPSGCTAERWAQCGGNGWSGCTTCVAGSTCTKINDWYHQCL

SEQ ID NO: 12 - DNA, 882 bp, Neurospora crassa
atgcgctcctccactattctgcaaaccgggctagtggccgctcttcctttcgccgtccaggctgcttccggatccggccagtccaccagatattgggactgctgcaaaccatcttgctcctggtccggcaaggctcctgtcaaccgacccgtcctcgcttgcgacgcaaacaacaaccccctgagcgacgccagtgtcaagtctggatgtgatggcggttctgcatacacctgtgccaacaactcaccatgggcggtgaacgaccagctctcctacggctttgccgccacgaaactcagtggtggaaccgagtcatcttggtgctgtgcctgttatgcccttaccttcacttcgggccctgttgctggcaagaccttggtcgttcagtctaccagtaccggcggtgatctcggctccaaccacttcgatatcaacatgcccggcggcggcgtcggcctgtttgatggatgtaaacgacagttcggcggtctccccggcgctcaatatggcggcatcagctcccgcagccagtgcgactcgttccctgccgctctcaagcccggttgccagtggcgcttcgactggttccagaacgccgataacccgaacttcaccttcaagcaggtccaatgcccatccgagctcacatcccgcaccggctgcaagcgaaacgacgactcccaattccctgtcttcactccgccctctggtggaggcagtaacccctctactccgacaacccctccctcttcaggcggcggttccggatgtacagcggataaatacgctcaatgtggtggctcggggtggtctggctgcaccaactgcccgtctggatcgacctgcaagactatcaacgattattaccatcagtgtgcctga

SEQ ID NO: 13 - protein, 293 aa, Neurospora crassa
MRSSTILQTGLVAALPFAVQAASGSGQSTRYWDCCKPSCSWSGKAPVNRPVLACDANNNPLSDASVKSGCDGGSAYTCANNSPWAVNDQLSYGFAATKLSGGTESSWCCACYALTFTSGPVAGKTLVVQSTSTGGDLGSNHFDINMPGGGVGLFDGCKRQFGGLPGAQYGGISSRSQCDSFPAALKPGCQWRFDWFQNADNPNFTFKQVQCPSELTSRTGCKRNDDSQFPVFTPPSGGGSNPSTPTTPPSSGGGSGCTADKYAQCGGSGWSGCTNCPSGSTCKTINDYYHQCA

SEQ ID NO: 14 - protein, 272 aa, Neurospora crassa
ASGSGQSTRYWDCCKPSCSWSGKAPVNRPVLACDANNNPLSDASVKSGCDGGSAYTCANNSPWAVNDQLSYGFAATKLSGGTESSWCCACYALTFTSGPVAGKTLVVQSTSTGGDLGSNHFDINMPGGGVGLFDGCKRQFGGLPGAQYGGISSRSQCDSFPAALKPGCQWRFDWFQNADNPNFTFKQVQCPSELTSRTGCKRNDDSQFPVFTPPSGGGSNPSTPTTPPSSGGGSGCTADKYAQCGGSGWSGCTNCPSGSTCKTINDYYHQCA

SEQ ID NO: 15 - DNA, 897 bp, Thielavia terrestris
atgcgctctactcccgttcttcgcacaaccctggccgctgcacttcctctggtcgcctccgcggccagtggcagtggccagtccacgagatactgggactgctgcaagccgtcgtgcgcttggcccgggaaggccgccgtcagccaaccggtctacgcgtgcgatgccaacttccagcgcctgtccgacttcaatgtccagtcgggctgcaacggcggctcggcctactcctgcgccgaccagactccctgggcggtgaacgacaatctcgcctacggcttcgccgcgacgagcatcgccggcgggtccgaatcctcgtggtgctgcgcctgctacgcgctcaccttcacttccggtcccgtcgccggcaagacaatggtggtgcagtcaacgagcactggcggcgacctgggaagtaaccatttcgatatcgccatgcccggcggcggcgtgggcatcttcaacggctgcagctcgcagttcggcggcctccccggcgctcaatacggcggcatttcgtcgcgcgaccagtgcgattccttccccgcgccgctcaagcccggctgccagtggcggtttgactggttccagaacgccgacaacccgacgttcacgttccagcaggtgcagtgccccgccgagatcgttgcccgctccggctgcaagcgcaacgacgactccagcttccccgtcttcacccccccaagcggtggcaacggtggcaccgggacgcccacgtcgactgcgcctgggtcgggccagacgtctcccggcggcggcagtggctgcacgtctcagaagtgggctcagtgcggtggcatcggcttcagcggatgcaccacctgtgtctctggcaccacctgccagaagttgaacgactactactcgcagtgcctc

SEQ ID NO: 16 - protein, 299 aa, Thielavia terrestris
MRSTPVLRTTLAAALPLVASAASGSGQSTRYWDCCKPSCAWPGKAAVSQPVYACDANFQRLSDFNVQSGCNGGSAYSCADQTPWAVNDNLAYGFAATSIAGGSESSWCCACYALTFTSGPVAGKTMVVQSTSTGGDLGSNHFDIAMPGGGVGIFNGCSSQFGGLPGAQYGGISSRDQCDSFPAPLKPGCQWRFDWFQNADNPTFTFQQVQCPAEIVARSGCKRNDDSSFPVFTPPSGGNGGTGTPTSTAPGSGQTSPGGGSGCTSQKWAQCGGIGFSGCTTCVSGTTCQKLNDYYSQCL

SEQ ID NO: 17 - protein, 278 aa, Thielavia terrestris [sequence omitted]

SEQ ID NO: 18 - protein, 305 aa, Thielavia hyrcaniae
MRSTPVLRTAIAAALPLVAFAADGKSTRYWDCCKPSCAWSGKAAVSAPVYACSANFQRLSDPNAKSGCDGGSAYTCADQTPWAINDNLSYGFAATSISGGSEASWCCACYELTFNSGPVAGKKMVVQSTSTGGDLGTNHFDLNIPGGGVGLFDGCKNQFGGLPGAQYGGISSRSQCDSFPEALKPGCYWRFDWFQNADNPTFTFRQVQCPSELVARTGCRRNDDSSFPVFTPGTSGSSSTAKPASSSTRATSTKTSAPATQTSSTGGGCVAQKWAQCGGSGFSGCTTCAAGSTCTKQNDYYSQCL

SEQ ID NO: 19 - protein, 293 aa, Chaetomium thermophilum
ADGKSTRYWDCCKPSCSWPGKAAVSQPVFACDRNFNRIYDFGAKSGCEGGPAYSCADQTPWAVNDQFSYGFAATNIAGGNEASWCCACYKLTFTSGPVAGKVMVVQSTSTGGDLGNNHFDLNIPGGGVGIFDGCTPQFGGLPGERYGGISSRSQCDSFPDALKPGCYWRFDWFLNADNPNFTFERVQCPSELVARTGCKRNDDGNYPVFTPPSGDSPSSSSAAPTSTSTSQQPQQPTSSSSQASVPTSNPGGCTSQKWAQCGGIGFTGCTTCVSGTTCTKLNDWYSQCTMINL

SEQ ID NO: 20 - protein, 235 aa, Melanocarpus albomyces
MRSTPVLRALLAAALPLGALAANGQSTRYWDCCKPSCGWRGKGPVNQPVYSCDANFQRIHDFDAVSGCEGGPAFSCADHSPWAINDNLSYGFAATALSGQTEESWCCACYALTFTSGPVAGKTMVVQSTSTGGDLGSNHFDLNIPGGGVGLFDGCTPQFGGLPGARYGGISSRQECDSFPEPLKPGCQWRFDWFQNADNPSFTFERVQCPEELVARTGCRRHDDGGFAVFKAPSA

SEQ ID NO: 21 - protein, 306 aa, unknown
  Humicola sp.
PFMMVAWWSLFLYGLQVAAPAFAADGRSTRYWDCCKPSCSWPGKALVNQPVYARNANFQRITDPNAKSGCDGGSAFSCADQTPWAVSDDFAYGFAATALAGQSESSWCCACYELTFTSGPVAGKKMAVQSTSTGGDLGSNHFDLNMPGGGVGIFDGCSPQVGGLAGQRYGGVSSRSECDSFPAALKPGCYWRYDWFKNADNPSFSFRQVQCPAELVARTGCRRNDDGNFPAVQIPSSSTSSPVNQPTSTSTTSTSTTSSPPVQPTTPSGCTAERWAQCGGNGWSGCTTCVAGSTCTKINDWYHQCL

SEQ ID NO: 22 - protein, 299 aa, Thielavia terrestris NRRL 8126
MRSTPVLRTTLAAALPLVASAASGSGQSTRYWDCCKPSCAWPGKAAVSQPVYACDANFQRLSDFNVQSGCNGGSAYSCADQTPWAVNDNLAYGFAATSIAGGSESSWCCACYALTFTSGPVAGKTMVVQSTSTGGDLGSNQFDIAMPGGGVGIFNGCSSQFGGLPGAQYGGISSRDQCDSFPAPLKPGCQWRFDWFQNADNPTFTFQQVQCPAEIVARSGCKRNDDSSFPVFTPPSGGNGGTGTPTSTAPGSGQTSPGGGSGCTSQKWAQCGGIGFSGCTTCVSGTTCQKLNDYYSQCL

SEQ ID NO: 23 - protein, 305 aa, Humicola grisea
MRSSPLLPSDVVAALPVLALAADGKSTRYWDCCKPSCGWAKKAPVNQPVFSCNANFQRLTDFDAKSGCEPGGVAYSCADQTPWAVNDDFAFGFAATSIAGSNEAGWCCACYELTFTSGPVAGKKMVVQSTSTGGDLGSNHFDLNIPGGGVGIFDGCTPQFGGLPGQRYGGISSRNECDRFPDALKPGCYWRFDWFKNADNPSFSFRQVQCPAELVARTGCRRNDDGNFPAVQIPSSSTSSPVGQPTSTSTTSTSTTSSPPVQPTTPSGCTAERWAQCGGNGWSGCTTCVAGSTCTKINDWYHQCL

SEQ ID NO: 24 - protein, 315 aa, unknown
  Acremonium sp.
MRSSPFLRAALAAALPLSAHALDGKSTRYWDCCKPSCGWAGKASVNQPVFSCSADWQRISDFNAKSGCDGGSAYSCADQTPWAVNDNFSYGFAATAIAGGSESSWCCACYALTFNSGPVAGKTMVVQSTSTGGDLGSNQFDLAIPGGGVGIFNGCASQFGGLPGAQYGGISDRSQCSSFPAPLQPGCQWRFDWFQNADNPTFTFQRVQCPSELTSRTGCKRDDDASYPVFNPPSVPGLDGSNPGNPTTTVVPPASTSTSRPTSSTSSPVSTPTGQPGGCTTQKWGQCGGIGYTGCTNCVAGTTCTQLNPWYSQCL

SEQ ID NO: 25 - protein, 302 aa, Podospora anserina
MRSSTVLQTSLLAVLPLAVQAQGASGSGKSTRYWDCCKPSCAWPGKAAVNRPVFACDANFQRISDSGVASGCNGGSAYSCADHSAWAINDNLSYGFAATALSGGSEASWCCACYELTFTDGPVAGKKMVVQSTSTGGDLGSNHFDLNIPGGGVGLFDGCKPQFGGLPGATYGGISDRSQCASFPDALKPGCNWRFDWFKNADNPSFTFRQVQCPSELTARSGCKRDDDSRFPVFSPPGGGSQPQPQPTSSAAQNPNPTPSAAPGGCRAAKYAQCGGQGFTGCTTCEAGSTCTASNQWYSQCL

SEQ ID NO: 26 - protein, 232 aa, Acremonium chrysogenum ATCC11550
MTPSVFKIALAAASVAAPALAAEGAGKSTRYWDCCKPSCAWPEKADVSAPAAVCNADNTPLNDPLADSGCDGGPAFTCANYSPWAVNDNLAYGFAATAINGGSEASWCCACYRLTFTDGPVAGKTMIVQSTNTGGDISNNHFDILMPGGGVGLFDGCTPQYGGIPGAQYGGVSSREECEQMPEALKEGCFWRFDWFANADNPNLNFEQVQCPSEITAISGCTRSDDGNFPAA

SEQ ID NO: 27 - protein, 304 aa, unknown
  Humicola sp.
MMVAWWSLFLYGLQVAAPAFAADGRSTRYWDCCKPSCAWSGKASVSSPVRTCDANNSPLSDVDAKSACDGGVAYTCSNNAPWAVNDNLSYGFAATAINGGSESSWCCACYKLTFTSGPASGKVMVVQSTNTGYDLSNNHFDILMPGGGVGAFDGCSRQYGSIPGERYGGVTSRDQCDQMPSALKQGCYWRFDWFKNADNPSFSFRQVQCPAELVARTGCRRNDDGNFPAVQIPSSSTSSPVNQPTSTSTTSTSTTSSPPVQPTTPSGCTAERWAQCGGNGWSGCTTCVAGSTCTKINDWYHQCL

SEQ ID NO: 28 - protein, 307 aa, unknown
  Humicola sp.
PFMMVAWWSLFLYGLQVAAPAFAADGRSTRYWDCCKPSCSWPDKAPVGSPVGTCDAGNSPLGDPLAKSGCEGGPSYTCANYQPWAVNDQLAYGFAATAINGGTEDSWCCACYKLTFTDGPASGKTMIVQSTNTGGDLSDNHFDLLIPGGGVGIFDGCTSQYGQALPGAQYGGVSSRAECDQMPEAIKAGCQWRYDWFKNADNPSFSFRQVQCPAELVARTGCRRNDDGNFPAVQIPSSSTSSPVNQPTSTSTTSTSTTSSPPVQPTTPSGCTAERWAQCGGNGWSGCTTCVAGSTCTKINDWYHQCL

SEQ ID NO: 29 - protein, 277 aa, Scytalidium indonesiacum
MRSSPLLRSAVVAALPVLALAADGKSTRYWDCCKPSCGWAKKAPVNQPVFSCNANFQRLYDFDAKSGCEPGGVAYSCADQTPWAVNDDFAFGFAATSIAGSNEAGWCCACYELTFTSGPVAGKKMVVQSTSTGGDLGSNHFDLNIPGGGVGIFDGCTPQFGGLPGQRYGGISSRNECERFPDALKPGCYWRFDWFKNADNPNFSFRQVQCPAELVARTGCRRNDDGNFPAVQIPSSSTSSPRIQNLGSTRMLSRSRRRRPAGGSQLAAAGGVRGGAP